European Patent Application EP 4 431 615 A1, published September 18, 2024. Title: Composition and method for preparing retinoids. Applicant: INDUSTRY-ACADEMIC COOPERATION FOUNDATION GYEONGSANG NATIONAL UNIVERSITY. Application KR. The sequence listing filed with the application follows.

SEQUENCE LISTING (74 sequences)

SEQ ID NO: 1 - protein, 275 aa, unidentified [sequence omitted]

SEQ ID NO: 2 - protein, 176 aa, Escherichia coli
MAITGIFFGSDTGNTENIAKMIQKQLGKDVADVHDIAKSSKEDLEAYDILLLGIPTWYYGEAQCDWDDFFPTLEEIDFNGKLVALFGCGDQEDYAEYFCDALGTIRDIIEPRGATIVGHWPTAGYHFEASKGLADDDHFVGLAIDEDRQPELTAERVEKWVKQISEELHLDEILNA

SEQ ID NO: 3 - protein, 173 aa, Escherichia coli
MNMGLFYGSSTCYTEMAAEKIRDIIGPELVTLHNLKDDSPKLMEQYDVLILGIPTWDFGEIQEDWEAVWDQLDDLNLEGKIVALYGLGDQLGYGEWFLDALGMLHDKLSTKGVKFVGYWPTEGYEFTSPKPVIADGQLFVGLALDETNQYDLSDERIQSWCEQILNEMAEHYA

SEQ ID NO: 4 - protein, 111 aa, Escherichia coli
MPKIVILPHQDLCPDGAVLEANSGETILDAALRNGIEIEHACEKSCACTTCHCIVREGFDSLPESSEQEDDMLDKAWGLEPESRLSCQARVTDEDLVVEIPRYTINHAREH

SEQ ID NO: 5 - protein, 248 aa, Escherichia coli
MADWVTGKVTKVQNWTDALFSLTVHAPVLPFTAGQFTKLGLEIDGERVQRAYSYVNSPDNPDLEFYLVTVPDGKLSPRLAALKPGDEVQVVSEAAGFFVLDEVPHCETLWMLATGTAIGPYLSILQLGKDLDRFKNLVLVHAARYAADLSYLPLMQELEKRYEGKLRIQTVVSRETAAGSLTGRIPALIESGELESTIGLPMNKETSHVMLCGNPQMVRDTQQLLKETRQMTKHLRRRPGHMTAEHYW

SEQ ID NO: 6 - protein, 1174 aa, Escherichia coli
MITIDGNGAVASVAFRTSEVIAIYPITPSSTMAEQADAWAGNGLKNVWGDTPRVVEMQSEAGAIATVHGALQTGALSTSFTSSQGLLLMIPTLYKLAGELTPFVLHVAARTVATHALSIFGDHSDVMAVRQTGCAMLCAANVQEAQDFALISQIATLKSRVPFIHFFDGFRTSHEINKIVPLADDTILDLMPQVEIDAHRARALNPEHPVIRGTSANPDTYFQSREATNPWYNAVYDHVEQAMNDFSAATGRQYQPFEYYGHPQAERVIILMGSAIGTCEEVVDELLTRGEKVGVLKVRLYRPFSAKHLLQALPGSVRSVAVLDRTKEPGAQAEPLYLDVMTALAEAFNNGERETLPRVIGGRYGLSSKEFGPDCVLAVFAELNAAKPKARFTVGIYDDVTNLSLPLPENTLPNSAKLEALFYGLGSDGSVSATKNNIKIIGNSTPWYAQGYFVYDSKKAGGLTVSHLRVSEQPIRSAYLISQADFVGCHQLQFIDKYQMAERLKPGGIFLLNTPYSADEVWSRLPQEVQAVLNQKKARFYVINAAKIARECGLAARINTVMQMAFFHLTQILPGDSALAELQGAIAKSYSSKGQDLVERNWQALALARESVEEVPLQPVNPHSANRPPVVSDAAPDFVKTVTAAMLAGLGDALPVSALPPDGTWPMGTTRWEKRNIAEEIPIWKEELCTQCNHCVAACPHSAIRAKVVPPEAMENAPASLHSLDVKSRDMRGQKYVLQVAPEDCTGCNLCVEVCPAKDRQNPEIKAINMMSRLEHVEEEKINYDFFLNLPEIDRSKLERIDIRTSQLITPLFEYSGACSGCGETPYIKLLTQLYGDRMLIANATGCSSIYGGNLPSTPYTTDANGRGPAWANSLFEDNAEFGLGFRLTVDQHRVRVLRLLDQFADKIPAELLTALKSDATPEVRREQVAALRQQLNDVAEAHELLRDADALVEKSIWLIGGDGWAYDIGFGGLDHVLSLTENVNILVLDTQCYSNTGGQASKATPLGAVTKFGEHGKRKARKDLGVSMMMYGHVYVAQISLGAQLNQTVKAIQEAEAYPGPSLIIAYSPCEEHGYDLALSHDQMRQLTATGFWPLYRFDPRRADEGKLPLALDSRPPSEAPEETLLHEQRFRRLNSQQPEVAEQLWKDAAADLQKRYDFLAQMAGKAEKSNTD

SEQ ID NO: 7 - DNA, 46 bp, synthetic construct
  misc_feature 1..46: note = FldA-Fwd
  source 1..46: mol_type = other DNA
attctagaaggaggtaataaatatggctatcactggcatctttttc

SEQ ID NO: 8 - DNA, 31 bp, synthetic construct
  misc_feature 1..31: note = FldA-Rev
  source 1..31: mol_type = other DNA
atgagctcttaggcattgagaatttcgtcga

SEQ ID NO: 9 - DNA, 49 bp, synthetic construct
  misc_feature 1..49: note = FldB-Fwd
  source 1..49: mol_type = other DNA
atggatccaggaggtaataaatatgaatatgggtcttttttacggttcc

SEQ ID NO: 10 - DNA, 30 bp, synthetic construct
  misc_feature 1..30: note = FldB-Rev
  source 1..30: mol_type = other DNA
attctagattaggcgtaatgctctgccatt

SEQ ID NO: 11 - DNA, 45 bp, synthetic construct
  misc_feature 1..45: note = Fdx-Fwd
  source 1..45: mol_type = other DNA
attctagaaggaggtaataaatatgccaaagattgttattttgcc

SEQ ID NO: 12 - DNA, 27 bp, synthetic construct
  misc_feature 1..27: note = Fdx-Rev
  source 1..27: mol_type = other DNA
atgagctcttaatgctcacgcgcatgg

SEQ ID NO: 13 - DNA, 43 bp, synthetic construct
  misc_feature 1..43: note = Fpr-Fwd
  source 1..43: mol_type = other DNA
atggtaccaggaggtaataaatatggctgattgggtaacaggc

SEQ ID NO: 14 - DNA, 30 bp, synthetic construct
  misc_feature 1..30: note = Fpr-Rev
  source 1..30: mol_type = other DNA
atgtcgacttaccagtaatgctccgctgtc

SEQ ID NO: 15 - DNA, 47 bp, synthetic construct
  misc_feature 1..47: note = YdbK-Fwd
  source 1..47: mol_type = other DNA
atgtcgacaggaggtaataaatatgattactattgacggtaatggcg

SEQ ID NO: 16 - DNA, 31 bp, synthetic construct
  misc_feature 1..31: note = YdbK1-Rev
  source 1..31: mol_type = other DNA
attctagattaatcggtgttgcttttttccg

SEQ ID NO: 17 - DNA, 31 bp, synthetic construct
  misc_feature 1..31: note = YdbK2-Rev
  source 1..31: mol_type = other DNA
ataagcttttaatcggtgttgcttttttccg

SEQ ID NO: 18 - protein, 803 aa, Enterococcus faecalis
LKTVVIIDALRTPIGKYKGSLSQVSAVDLGTHVTTQLLKRHSTISEEIDQVIFGNVLQAGNGQNPARQIAINSGLSHEIPAMTVNEVCGSGMKAVILAKQLIQLGEAEVLIAGGIENMSQAPKLQRFNYETESYDAPFSSMMYDGLTDAFSGQAMGLTAENVAEKYHVTREEQDQFSVHSQLKAAQAQAEGIFADEIAPLEVSGTLVEKDEGIRPNSSVEKLGTLKTVFKEDGTVTAGNASTINDGASALIIASQEYAEAHGLPYLAIIRDSVEVGIDPAYMGISPIKAIQKLLARNQLTTEEIDLYEINEAFAATSIVVQRELALPEEKVNIYGGGISLGHAIGATGARLLTSLSYQLNQKEKKYGVASLCIGGGLGLAMLLERPQQKKNSRFYQMSPEERLASLLNEGQISADTKKEFENTALSSQIANHMIENQISETEVPMGVGLHLTVDETDYLVPMATEEPSVIAALSNGAKIAQGFKTVNQQRLMRGQIVFYDVADAESLIDELQVRETEIFQQAELSYPSIVKRGGGLRDLQYRAFDESFVSVDFLVDVKDAMGANIVNAMLEGVAELFREWFAEQKILFSILSNYATESVVTMKTAIPVSRLSKGSNGREIAEKIVLASRYASLDPYRAVTHNKGIMNGIEAVVLATGNDTRAVSASCHAFAVKEGRYQGLTSWTLDGEQLIGEISVPLALATVGGATKVLPKSQAAADLLAVTDAKELSRVVAAVGLAQNLAALRALVSEGIQKGHMALQARSLAMTVGATGKEVEAVAQQLKRQKTMNQDRALAILNDLRKQ

SEQ ID NO: 19 - protein, 383 aa, Enterococcus faecalis
MTIGIDKISFFVPPYYIDMTALAEARNVDPGKFHIGIGQDQMAVNPISQDIVTFAANAAEAILTKEDKEAIDMVIVGTESSIDESKAAAVVLHRLMGIQPFARSFEIKEACYGATAGLQLAKNHVALHPDKKVLVVAADIAKYGLNSGGEPTQGAGAVAMLVASEPRILALKEDNVMLTQDIYDFWRPTGHPYPMVDGPLSNETYIQSFAQVWDEHKKRTGLDFADYDALAFHIPYTKMGKKALLAKISDQTEAEQERILARYEESIIYSRRVGNLYTGSLYLGLISLLENATTLTAGNQIGLFSYGSGAVAEFFTGELVAGYQNHLQKETHLALLDNRTELSIAEYEAMFAETLDTDIDQTLEDELKYSISAINNTVRSYRN

SEQ ID NO: 20 - protein, 292 aa, Streptococcus pneumoniae
MTKKVGVGQAHSKIILIGEHAVVYGYPAISLPLLEVEVTCKVVPAESPWRLYEEDTLSMAVYASLEYLNITEACIRCEIDSAIPEKRGMGSSAAISIAAIRAVFDYYQADLPHDVLEILVNRAEMIAHMNPSGLDAKTCLSDQPIRFIKNVGFTELEMDLSAYLVIADTGVYGHTREAIQVVQNKGKDALPFLHALGELTQQAEVAISQKDAEGLGQILSQAHLHLKEIGVSSPEADFLVETTLSHGALGAKMSGGGLGGCIIALVTNLTHAQELAERLEEKGAVQTWIESL

SEQ ID NO: 21 - protein, 336 aa, Streptococcus pneumoniae
MIAVKTCGKLYWAGEYAILEPGQLALIKDIPIYMRAEIAFSDSYRIYSDMFDFAVDLRPNPDYSLIQETIALMGDFLAVRGQNLRPFSLKICGKMEREGKKFGLGSSGSVVVLVVKALLALYNLSVDQNLLFKLTSAVLLKRGDNGSMGDLACIVAEDLVLYQSFDRQKAAAWLEEENLATVLERDWGFFISQVKPTLECDFLVGWTKEVAVSSHMVQQIKQNINQNFLSSSKETVVSLVEALEQGKAEKVIEQVEVASKLLEGLSTDIYTPLLRQLKEASQDLQAVAKSSGAGGGDCGIALSFDAQSSRNTLKNRWADLGIELLYQERIGHDDKS

SEQ ID NO: 22 - protein, 317 aa, Streptococcus pneumoniae
MDREPVTVRSYANIAIIKYWGKKKEKEMVPATSSISLTLENMYTETTLSPLPANVTADEFYINGQLQNEVEHAKMSKIIDRYRPAGEGFVRIDTQNNMPTAAGLSSSSSGLSALVKACNAYFKLGLDRSQLAQEAKFASGSSSRSFYGPLGAWDKDSGEIYPVETDLKLAMIMLVLEDKKKPISSRDGMKLCVETSTTFDDWVRQSEKDYQDMLIYLKENDFAKIGELTEKNALAMHATTKTASPAFSYLTDASYEAMAFVRQLREKGEACYFTMDAGPNVKVFCQEKDLEHLSEIFGQRYRLIVSKTKDLSQDDCC

SEQ ID NO: 23 - protein, 182 aa, Escherichia coli
MQTEHVILLNAQGVPTGTLEKYAAHTADTRLHLAFSSWLFNAKGQLLVTRRALSKKAWPGVWTNSVCGHPQLGESNEDAVIRRCRYELGVEITPPESIYPDFRYRATDPSGIVENEVCPVFAARTTSALQINDDEVMDYQWCDLADVLHGIDATPWAFSPWMVMQATNREARKRLSAFTQLK

SEQ ID NO: 24 - DNA, 35 bp, synthetic construct
  misc_feature 1..35: note = EFAES-F
  source 1..35: mol_type = other DNA
gccccgggtaggaaacagaccatggagttgaaaac

SEQ ID NO: 25 - DNA, 33 bp, synthetic construct
  misc_feature 1..33: note = EFAES-R
  source 1..33: mol_type = other DNA
cgcctgcaggttagtttcgataagagcgaacgg

SEQ ID NO: 26 - DNA, 74 bp, synthetic construct
  misc_feature 1..74: note = IS ackA-pta-Ptrc-F
  source 1..74: mol_type = other DNA
tggctccctgacgtttttttagccacgtatcaattataggtacttccatggtttgacagcttatcatcgactgc

SEQ ID NO: 27 - DNA, 70 bp, synthetic construct
  misc_feature 1..70: note = KO ackA-pta-R
  source 1..70: mol_type = other DNA
gcagcgcaaagctgcggatgatgacgagattactgctgctgtgcagactgtgtaggctggagctgcttcg

SEQ ID NO: 28 - DNA, 20 bp, synthetic construct
  misc_feature 1..20: note = KOackA-ptaCF-F
  source 1..20: mol_type = other DNA
tgtcatcatgcgctacgctc

SEQ ID NO: 29 - DNA, 20 bp, synthetic construct
  misc_feature 1..20: note = KOackA-ptaCF-R
  source 1..20: mol_type = other DNA
cagttaagcaagataatcag

SEQ ID NO: 30 - DNA, 46 bp, synthetic construct
  misc_feature 1..46: note = SN12Didi-F
  source 1..46: mol_type = other DNA
gcgaattcaggaggtaataatatgacaaaaaaagttggtgtcggtc

SEQ ID NO: 31 - DNA, 39 bp, synthetic construct
  misc_feature 1..39: note = SN12Didi-R
  source 1..39: mol_type = other DNA
cgcctgcaggttatttaagctgggtaaatgcagataatc

SEQ ID NO: 32 - DNA, 74 bp, synthetic construct
  misc_feature 1..74: note = IS poxB-Ptrc-F
  source 1..74: mol_type = other DNA
gatgaactaaacttgttaccgttatcacattcaggagatggagaaccatggtttgacagcttatcatcgactgc

SEQ ID NO: 33 - DNA, 70 bp, synthetic construct
  misc_feature 1..70: note = KO poxB -R
  source 1..70: mol_type = other DNA
ccttattatgacgggaaatgccaccctttttaccttagccagtttgtttttgtaggctggagctgcttcg

SEQ ID NO: 34 - DNA, 74 bp, synthetic construct
  misc_feature 1..74: note = IS ldhA-Ptrc-F
  source 1..74: mol_type = other DNA
atttttagtagcttaaatgtgattcaacatcactggagaaagtcttatgagtttgacagcttatcatcgactgc

SEQ ID NO: 35 - DNA, 70 bp, synthetic construct
  misc_feature 1..70: note = KO ldhA-R
  source 1..70: mol_type = other DNA
ctcccctggaatgcaggggagcggcaagattaaaccagttcgttcgggcatgtaggctggagctgcttcg

SEQ ID NO: 36 - DNA, 74 bp, synthetic construct
  misc_feature 1..74: note = IS adhE-Ptrc-F
  source 1..74: mol_type = other DNA
cgagcagatgatttactaaaaaagtttaacattatcaggagagcattatggtttgacagcttatcatcgactgc

SEQ ID NO: 37 - DNA, 70 bp, synthetic construct
  misc_feature 1..70: note = KO adhE-R
  source 1..70: mol_type = other DNA
ccgtttatgttgccagacagcgctactgattaagcggattttttcgcttttgtaggctggagctgcttcg

SEQ ID NO: 38 - DNA, 74 bp, synthetic construct
  misc_feature 1..74: note = IS atoDA-Ptrc-F5
  source 1..74: mol_type = other DNA
ctattgcctgactgtacccacaacggtgtatgcaagagggataaaaaatggtttgacagcttatcatcgactgc

SEQ ID NO: 39 - DNA, 70 bp, synthetic construct
  misc_feature 1..70: note = KO atoDA-R
  source 1..70: mol_type = other DNA
acgcgtcataaaacgcgatatgcgaccaatcataaatcaccccgttgcgttgtaggctggagctgcttcg

SEQ ID NO: 40 - DNA, 22 bp, synthetic construct
  misc_feature 1..22: note = KOpoxBCF-F
  source 1..22: mol_type = other DNA
ttacgtactggcctgctcctgc

SEQ ID NO: 41 - DNA, 22 bp, synthetic construct
  misc_feature 1..22: note = KOpoxBCF-R
  source 1..22: mol_type = other DNA
gtcgggtaacggtatcactgcg

SEQ ID NO: 42 - DNA, 20 bp, synthetic construct
  misc_feature 1..20: note = KOldhACF-F
  source 1..20: mol_type = other DNA
tcatcagcagcgtcaacggc

SEQ ID NO: 43 - DNA, 20 bp, synthetic construct
  misc_feature 1..20: note = KOldhACF-R
  source 1..20: mol_type = other DNA
cgctggtcacgggcttaccg

SEQ ID NO: 44 - DNA, 20 bp, synthetic construct
  misc_feature 1..20: note = KOadhECF-F
  source 1..20: mol_type = other DNA
ccgcactgactatactctcg

SEQ ID NO: 45 - DNA, 20 bp, synthetic construct
  misc_feature 1..20: note = KOadhECF-R
  source 1..20: mol_type = other DNA
tgatcggcattgcccagaag

SEQ ID NO: 46 - DNA, 22 bp, synthetic construct
  misc_feature 1..22: note = KOatoDACF-F
  source 1..22: mol_type = other DNA
ctggcgaggtaaaaacagcccc

SEQ ID NO: 47 - DNA, 22 bp, synthetic construct
  misc_feature 1..22: note = KOatoDACF-R
  source 1..22: mol_type = other DNA
aagcgcgatcacgaatgttagc

SEQ ID NO: 48 - protein, 307 aa, unidentified
  REGION 1..307: note = pantoea agglomerans crtE
MVSGSKAGVSPHREIEVMRQSIDDHLAGLLPETDSQDIVSLAMREGVMAPGKRIRPLLMLLAARDLRYQGSMPTLLDLACAVELTHTASLMLDDMPCMDNAELRRGQPTTHKKFGESVAILASVGLLSKAFGLIAATGDLPGERRAQAVNELSTAVGVQGLVLGQFRDLNDAALDRTPDAILSTNHLKTGILFSAMLQIVAIASASSPSTRETLHAFALDFGQAFQLLDDLRDDHPETGKDRNKDAGKSTLVNRLGADAARQKLREHIDSADKHLTFACPQGGAIRQFMHLWFGHHLADWSPVMKIA

SEQ ID NO: 49 - protein, 309 aa, unidentified
  REGION 1..309: note = pantoea agglomerans crtB
MSQPPLLDHATQTMANGSKSFATAAKLFDPATRRSVLMLYTWCRHCDDVIDDQTHGFASEAAAEEEATQRLARLRTLTLAAFEGAEMQDPAFAAFQEVALTHGITPRMALDHLDGFAMDVAQTRYVTFEDTLRYCYHVAGVVGLMMARVMGVRDERVLDRACDLGLAFQLTNIARDIIDDAAIDRCYLPAEWLQDAGLTPENYAARENRAALARVAERLIDAAEPYYISSQAGLHDLPPRCAWAIATARSVYREIGIKVKAAGGSAWDRRQHTSKGEKIAMLMAAPGQVIRAKTTRVTPRPAGLWQRPV

SEQ ID NO: 50 - protein, 492 aa, unidentified
  REGION 1..492: note = pantoea agglomerans crtI
MKKTVVIGAGFGGLALAIRLQAAGIPTVLLEQRDKPGGRAYVWHDQGFTFDAGPTVITDPTALEALFTLAGRRMEDYVRLLPVKPFYRLCWESGKTLDYANDSAELEAQITQFNPRDVEGYRRFLAYSQAVFQEGYLRLGSVPFLSFRDMLRAGPQLLKLQAWQSVYQSVSRFIEDEHLRQAFSFHSLLVGGNPFTTSSIYTLIHALEREWGVWFPEGGTGALVNGMVKLFTDLGGEIELNARVEELVVADNRVSQVRLADGRIFDTDAVASNADVVNTYKKLLGHHPVGQKRAAALERKSMSNSLFVLYFGLNQPHSQLAHHTICFGPRYRELIDEIFTGSALADDFSLYLHSPCVTDPSLAPPGCASFYVLAPVPHLGNAPLDWAQEGPKLRDRIFDYLEERYMPGLRSQLVTQRIFTPADFHDTLDAHLGSAFSIEPLLTQSAWFRPHNRDSDIANLYLVGAGTHPGAGIPGVVASAKATASLMIEDLQ

SEQ ID NO: 51 - protein, 382 aa, unidentified
  REGION 1..305: note = pantoea agglomerans crtY
MQPHYDLILVGAGLANGLIALRLQQQQPDMRILLIDAAPQAGGNHTWSFHHDDLTESQHRWIAPLVVHHWPDYQVRFPTRRRKLNSGYFCITSQRFAEVLQRQFGPHLWMDTAVAEVNAESVRLKKGQVIGARAVIDGRGYAANSALSVGFQAFIGQEWRLSHPHGLSSPIIMDATVDQQNGYRFVYSLPLSPTRLLIEDTHYIDNATLDPECARQNICDYAAQQGWQLQTLLREEQGALPITLSGNADAFWQQRPLACSGLRAGLFHPTTGYSLPLAVAVADRLSALDVFTSASIHHAITHFARERWQQQGFFRMLNRMLFLAGPADSRWRVMQRFYGLPEDLIARFYAGKLTLTDRLRILSGKPPVPVLAALQAIMTTHR

SEQ ID NO: 52 - protein, 305 aa, Haematococcus pluvialis
MLRSLLRGLTHIPRVNSAQQPSCAHARLQFKLRSMQMTLMQPSISANLSRAEDRTDHMRGASTWAGGQSQDELMLKDECILVDVEDNITGHASKLECHKFLPHQPAGLLHRAFSVFLFDDQGRLLLQQRARSKITFPSVWTNTCCSHPLHGQTPDEVDQLSQVADGTVPGAKAAAIRKLEHELGIPAHQLPASAFRFLTRLHYCAADVQPAATQSALWGEHEMDYILFIRANVTLAPNPDEVDEVRYVTQEELRQMMQPDNGLQWSPWFRIIAARFLERWWADLDAALNTDKHEDWGTVHHINEA

SEQ ID NO: 53 - DNA, 33 bp, synthetic construct
  misc_feature 1..33: note = LYCm4-F
  source 1..33: mol_type = other DNA
cgtacatgtgtttgacagcttatcatcgactgc

SEQ ID NO: 54 - DNA, 30 bp, synthetic construct
  misc_feature 1..30: note = LYCm4-R
  source 1..30: mol_type = other DNA
gctgatatcgggttattgtctcatgagcgg

SEQ ID NO: 55 - DNA, 74 bp, synthetic construct; identical to SEQ ID NO: 32
  misc_feature 1..74: note = IS poxB-Ptrc-F
  source 1..74: mol_type = other DNA

SEQ ID NO: 56 - DNA, 70 bp, synthetic construct; identical to SEQ ID NO: 33
  misc_feature 1..70: note = KO poxB -R
  source 1..70: mol_type = other DNA

SEQ ID NO: 57 - DNA, 74 bp, synthetic construct; identical to SEQ ID NO: 34
  misc_feature 1..74: note = IS ldhA-Ptrc-F
  source 1..74: mol_type = other DNA

SEQ ID NO: 58 - DNA, 70 bp, synthetic construct; identical to SEQ ID NO: 35
  misc_feature 1..70: note = KO ldhA-R
  source 1..70: mol_type = other DNA

SEQ ID NO: 59 - DNA, 74 bp, synthetic construct
  misc_feature 1..74: note = IS dld-Ptrc-F
  source 1..74: mol_type = other DNA
cgctattctagtttgtgatattttttcgccaccacaaggagtggaaaatggtttgacagcatcatcgactgctt

SEQ ID NO: 60 - DNA, 70 bp, synthetic construct
  misc_feature 1..70: note = KO dld-R
  source 1..70: mol_type = other DNA
ggatggcgatactctgccatccgtaatttttactccacttcctgccagtttgtaggctggagctgcttcg

SEQ ID NO: 61 - DNA, 74 bp, synthetic construct; identical to SEQ ID NO: 38
  misc_feature 1..74: note = IS atoDA-Ptrc-F
  source 1..74: mol_type = other DNA

SEQ ID NO: 62 - DNA, 70 bp, synthetic construct; identical to SEQ ID NO: 39
  misc_feature 1..70: note = KO atoDA-R
  source 1..70: mol_type = other DNA

SEQ ID NO: 63 - DNA, 74 bp, synthetic construct
  misc_feature 1..74: note = IS pps-Ptrc-F
  source 1..74: mol_type = other DNA
agaaatgtgtttctcaaaccgttcatttatcacaaaaggattgttcgatggtttgacagcttatcatcgactgc

SEQ ID NO: 64 - DNA, 70 bp, synthetic construct
  misc_feature 1..70: note = KO pps-R
  source 1..70: mol_type = other DNA
cggcgactaaacgccgccggggatttattttatttcttcagttcagccagtgtaggctggagctgcttcg

SEQ ID NO: 65 - DNA, 22 bp, synthetic construct
  misc_feature 1..22: note = KOpoxBCF-F
  source 1..22: mol_type = other DNA
ttacgtactggcctgctcctgc

SEQ ID NO: 66 - DNA, 22 bp, synthetic construct
  misc_feature 1..22: note = KOpoxBCF-R
  source 1..22: mol_type = other DNA
gtcgggtaacggtatcactgcg

SEQ ID NO: 67 - DNA, 20 bp, synthetic construct
  misc_feature 1..20: note = KOldhACF-F
  source 1..20: mol_type = other DNA
tcatcagcagcgtcaacggc

SEQ ID NO: 68 - DNA, 20 bp, synthetic construct
  misc_feature 1..20: note = KOldhACF-R
  source 1..20: mol_type = other DNA
cgctggtcacgggcttaccg

SEQ ID NO: 69 - DNA, 23 bp, synthetic construct
  misc_feature 1..23: note = KOdldCF-F
  source 1..23: mol_type = other DNA
cagactcaccgcgattcctactg

SEQ ID NO: 70 - DNA, 21 bp, synthetic construct
  misc_feature 1..21: note = KOdldCF-R
  source 1..21: mol_type = other DNA
cggtaaagtgatgcctgtgcc

SEQ ID NO: 71 - DNA, 22 bp, synthetic construct
  misc_feature 1..22: note = KOatoDACF-F
  source 1..22: mol_type = other DNA
ctggcgaggtaaaaacagcccc

SEQ ID NO: 72 - DNA, 22 bp, synthetic construct
  misc_feature 1..22: note = KOatoDACF-R
  source 1..22: mol_type = other DNA
aagcgcgatcacgaatgttagc

SEQ ID NO: 73 - DNA, 20 bp, synthetic construct
  misc_feature 1..20: note = KOppsCF-F
  source 1..20: mol_type = other DNA
gcagatttgcgcaacgctgg

SEQ ID NO: 74 - DNA, 21 bp, synthetic construct
  misc_feature 1..21: note = KOppsCF-R
  source 1..21: mol_type = other DNA
ctgccgtatggatgaggctgg